European Patent Application EP 4 166 672 A1, published April 19, 2023. Title: A novel method for purification of protein- or peptide-based capsules. Applicant: NEUWAY Pharma GmbH. The sequence listing filed with the application follows.

SEQUENCE LISTING (4 sequences)

SEQ ID NO: 1 - protein, 354 aa, Artificial Sequence
  derived from JC virus
MAPTKRKGEPKDPVQVPKLLIRGGVEVLEVKTGVDSITEVECFLTPEMGDPDEHLRGFSKSISISDTFESDSPNRDMLPCYSVARIPLPNLNEDLTCGNILMWEAVTLKTEVIGVTSLMNVHSNGQATHDNGAGKPVQGTSFHFFSVGGEALELQGVVFNYRTKYPDGTIFPKNATVQSQVMNTEHKAYLDKNKAYPVECWVPDPTRNENTRYFGTLTGGENVPPVLHITNTATTVLLDEFGVGPLCKGDNLYLSAVDVCGMFTNRSGSQQWRGLSRYFKVQLRKRRVKNPYPISFLLTDLINRRTPRVDGQPMYGMDAQVEEVRVFEGTEELPGDPDMMRYVDKYGQLQTKML

SEQ ID NO: 2 - DNA, 1065 bp, Artificial Sequence
  derived from JC virus
atggctcccaccaagcgcaagggcgagcccaaggaccccgtgcaagtgcccaagctgctgatccgtggtggtgtcgaggtgctggaagtcaagaccggcgtggactccattaccgaggtggagtgcttcctcacccccgagatgggtgaccctgacgagcacctgaggggcttctccaagtccatctccatctccgacaccttcgagtccgactcccccaaccgtgacatgctgccctgctactccgtggctcgtatccccctgcccaacctgaacgaggacctgacttgcggcaacatcctgatgtgggaggctgtgaccctcaagaccgaggtcatcggcgtgacttccctgatgaacgtgcactccaacggccaggctacccacgacaacggtgctggcaagcccgtgcagggaacctccttccacttcttctccgtgggtggcgaggctctggaactccagggcgtggtgttcaactaccgtaccaagtaccccgacggcaccatcttccccaagaacgctactgtgcagtcccaagtgatgaacaccgagcacaaggcttacctggacaagaacaaggcctaccccgtggagtgctgggtgcccgaccccacccgtaacgagaacacccgttacttcggcaccctgaccggtggagagaacgtgccccccgtgctgcacatcaccaacaccgctaccaccgtgctgctggacgagttcggtgtcggtcccctgtgcaagggcgacaacctgtacctgtccgctgtggacgtgtgcggcatgttcaccaaccgttccggttcccagcagtggcgtggcctgtcccgctacttcaaggtgcagctgcgcaagcgtcgtgtgaagaacccctaccctatctccttcctgctgaccgacctgatcaaccgtcgtacccctcgtgtggacggccagcccatgtacggcatggacgctcaggtggaagaggtccgcgtgttcgagggcaccgaggaattgcccggcgaccccgacatgatgcgttacgtggacaagtacggccagctccagaccaagatgctgtaa

SEQ ID NO: 3 - protein, 354 aa, JC virus
MAPTKRKGERKDPVQVPKLLIRGGVEVLEVKTGVDSITEVECFLTPEMGDPDEHLRGFSKSISISDTFESDSPSKDMLPCYSVARIPLPNLNEDLTCGNILMWEAVTLKTEVIGVTSLMNVHSNGQAAHDNGAGKPVQGTSFHFFSVGGEALELQGVVFNYRTKYPDGTIFPKNATVQSQVMNTEHKAYLDKNKAYPVECWVPDPTRNENTRYFGTLTGGENVPPVLHITNTATTVLLDEFGVGPLCKGDNLYLSAVDVCGMFTNRSGSQQWRGLSRYFKVQLRKRRVKNPYPISFLLTDLINRRTPRVDGQPMYGMDAQVEEVRVFEGTEELPGDPDMMRYVDRYGQLQTKML

SEQ ID NO: 4 - DNA, 1065 bp, JC virus
atggccccaacaaaaagaaaaggagaaaggaaggaccccgtgcaagttccaaaacttcttataagaggaggagtagaagttctagaagttaaaactggggttgactcaattacagaggtagaatgctttttaactccagaaatgggtgacccagatgagcatcttaggggttttagtaagtcaatatctatatcagatacatttgaaagtgactccccaaatagggacatgcttccttgttacagtgtggccagaattccactacccaatctaaatgaggatctaacctgtggaaatatactcatgtgggaggctgtgaccttaaaaactgaggttataggggtgacaagtttgatgaatgtgcactctaatgggcaagcaactcatgacaatggtgcagggaagccagtgcagggcaccagctttcattttttttctgttgggggggaggctttagaattacagggggtgctttttaattacagaacaaagtacccagatggaacaatttttccaaagaatgccacagtgcaatctcaagtcatgaacacagagcacaaggcgtacctagataagaacaaagcatatcctgttgaatgttgggttcctgatcccaccagaaatgaaaacacaagatattttgggacactaacaggaggagaaaatgttcctccagttcttcatataacaaacactgccacaacagtgttgcttgatgaatttggtgttgggccactttgcaaaggtgacaacttatacttgtcagctgttgatgtctgtggcatgtttacaaacaggtctggttcccagcagtggagaggactctccagatattttaaggtgcagctaaggaaaaggagggttaaaaacccctacccaatttctttccttcttactgatttaattaacagaaggactcctagagttgatgggcagcctatgtatggcatggatgctcaagtagaggaggttagagtttttgagggaacagaggagcttccaggggacccagacatgatgagatacgttgacaaatatggacagttgcagacaaaaatgctgtaa